European Patent Application EP 4 159 759 A1, published April 5, 2023. Title: Anti-B7-H3 antibody and preparation thereof and use thereof. Applicant: MINGHUI PHARMACEUTICAL (SHANGHAI) LIMITED MINGHUI PHARMACEUTICAL (HANGZHOU) LIMITED. The sequence listing filed with the application follows.

SEQUENCE LISTING (97 sequences)

SEQ ID NO: 1 - protein, 11 aa, Mus musculus
RASENIYSNLA

SEQ ID NO: 2 - protein, 7 aa, Mus musculus
AATNLAD

SEQ ID NO: 3 - protein, 10 aa, Mus musculus
QHFWGTPPWT

SEQ ID NO: 4 - protein, 12 aa, Mus musculus
SASSSISSNYLH

SEQ ID NO: 5 - protein, 7 aa, Mus musculus
STSNLAS

SEQ ID NO: 6 - protein, 9 aa, Mus musculus
QQYSGYPLT

SEQ ID NO: 7 - protein, 11 aa, Mus musculus
KASQNVGTNVA

SEQ ID NO: 8 - protein, 7 aa, Mus musculus
SASYRYS

SEQ ID NO: 9 - protein, 9 aa, Mus musculus
QQYNSYPYT

SEQ ID NO: 10 - protein, 10 aa, Mus musculus
SASSSISYMH

SEQ ID NO: 11 - protein, 7 aa, Mus musculus
DTSKLAS

SEQ ID NO: 12 - protein, 9 aa, Mus musculus
QQWSSNPLT

SEQ ID NO: 13 - protein, 11 aa, Mus musculus
RASENIYSYLA

SEQ ID NO: 14 - protein, 7 aa, Mus musculus
NAKTLAE

SEQ ID NO: 15 - protein, 10 aa, Mus musculus
QHHYGTPPYT

SEQ ID NO: 16 - protein, 11 aa, Mus musculus
KASQNVGTNVA

SEQ ID NO: 17 - protein, 7 aa, Mus musculus
SASYRYS

SEQ ID NO: 18 - protein, 9 aa, Mus musculus
QQYNSYPYT

SEQ ID NO: 19 - protein, 11 aa, Mus musculus
KASQNVGTAVA

SEQ ID NO: 20 - protein, 7 aa, Mus musculus
SASNRYT

SEQ ID NO: 21 - protein, 9 aa, Mus musculus
QQYSSYPFT

SEQ ID NO: 22 - protein, 11 aa, Mus musculus
RASQSVSTYLA

SEQ ID NO: 23 - protein, 7 aa, Mus musculus
DASNRAT

SEQ ID NO: 24 - protein, 11 aa, Mus musculus
QQRSNWPPLFT

SEQ ID NO: 25 - protein, 7 aa, Artificial Sequence
  CDR of light chain variable region
AATNLQS

SEQ ID NO: 26 - protein, 7 aa, Artificial Sequence
  CDR of light chain variable region
AASNLQS

SEQ ID NO: 27 - protein, 12 aa, Artificial Sequence
  CDR of light chain variable region
RASSSISSNYLH

SEQ ID NO: 28 - protein, 7 aa, Artificial Sequence
  CDR of light chain variable region
STSNLQS

SEQ ID NO: 29 - protein, 10 aa, Mus musculus
SASSSVSYMH

SEQ ID NO: 30 - protein, 11 aa, Mus musculus
RASQSVSSYLA

SEQ ID NO: 31 - protein, 11 aa, Mus musculus
QQRSNWPPSLT

SEQ ID NO: 32 - protein, 11 aa, Mus musculus
QQRSNWPPMYT

SEQ ID NO: 33 - protein, 10 aa, Mus musculus
GFTFSSYGMS

SEQ ID NO: 34 - protein, 10 aa, Mus musculus
TINSNGGTTY

SEQ ID NO: 35 - protein, 10 aa, Mus musculus
NEEFRRGLAY

SEQ ID NO: 36 - protein, 10 aa, Mus musculus
GYTFTDYAIH

SEQ ID NO: 37 - protein, 10 aa, Mus musculus
IINTYNGNSN

SEQ ID NO: 38 - protein, 12 aa, Mus musculus
NYGSSFNWYFDV

SEQ ID NO: 39 - protein, 10 aa, Mus musculus
GYTFTDYVIH

SEQ ID NO: 40 - protein, 10 aa, Mus musculus
GINRDSGGTT

SEQ ID NO: 41 - protein, 9 aa, Mus musculus
WKFPWYFDV

SEQ ID NO: 42 - protein, 10 aa, Mus musculus
GFTFSSYGMS

SEQ ID NO: 43 - protein, 10 aa, Mus musculus
TISGGGRYTY

SEQ ID NO: 44 - protein, 8 aa, Mus musculus
HYDGYLDY

SEQ ID NO: 45 - protein, 10 aa, Mus musculus
GDSITSGSWN

SEQ ID NO: 46 - protein, 9 aa, Mus musculus
YISYSGSIY

SEQ ID NO: 47 - protein, 8 aa, Mus musculus
GNPAWFAY

SEQ ID NO: 48 - protein, 10 aa, Mus musculus
GYTFTDYAMH

SEQ ID NO: 49 - protein, 10 aa, Mus musculus
IINTYNGNTN

SEQ ID NO: 50 - protein, 11 aa, Mus musculus
SRGPWDRYFDV

SEQ ID NO: 51 - protein, 10 aa, Mus musculus
GGTFSSYAIS

SEQ ID NO: 52 - protein, 10 aa, Mus musculus
GIIPILGIAN

SEQ ID NO: 53 - protein, 9 aa, Mus musculus
GDSGYDSNY

SEQ ID NO: 54 - protein, 10 aa, Artificial Sequence
  CDR of heavy chain variable region
AINSNGGSTY

SEQ ID NO: 55 - protein, 10 aa, Mus musculus
VINTYSGNTN

SEQ ID NO: 56 - protein, 15 aa, Mus musculus
GVTYGSGYPYWYFDV

SEQ ID NO: 57 - protein, 10 aa, Mus musculus
GYTFTEYVIH

SEQ ID NO: 58 - protein, 10 aa, Mus musculus
GGSGRYLPDY

SEQ ID NO: 59 - protein, 10 aa, Mus musculus
GIIPIFGTAN

SEQ ID NO: 60 - protein, 10 aa, Mus musculus
GERGSYLIDY

SEQ ID NO: 61 - protein, 108 aa, Mus musculus
DIQMIQSPASLSVSVGETVTITCRASENIYSNLAWYQQKQGKSPQLLVYAATNLADGVPSRFSGSGSGTQYSLKINSLQSEDFGSYYCQHFWGTPPWTFGGGTKLEIK

SEQ ID NO: 62 - protein, 108 aa, Artificial Sequence
  Humanized light chain variable region
DIQMTQSPSSLSASVGDRVTITCRASENIYSNLAWYQQKPGKAPKLLVYAATNLADGVPSRFSGSGSGTDYTLTISSLQPEDFATYYCQHFWGTPPWTFGQGTKLEIK

SEQ ID NO: 63 - protein, 108 aa, Artificial Sequence
  Humanized light chain variable region
DIQMTQSPSSLSASVGDRVTITCRASENIYSNLAWYQQKPGKAPKLLVYAATNLQSGVPSRFSGSGSGTDYTLTISSLQPEDFATYYCQHFWGTPPWTFGQGTKLEIK

SEQ ID NO: 64 - protein, 108 aa, Artificial Sequence
  Humanized light chain variable region
DIQMTQSPSSLSASVGDRVTITCRASENIYSNLAWYQQKPGKAPKLLIYAASNLQSGVPSRFSGSGSGTDYTLTISSLQPEDFATYYCQHFWGTPPWTFGQGTKLEIK

SEQ ID NO: 65 - protein, 108 aa, Mus musculus
DIVLTQSPTTMAASPGEKITITCSASSSISSNYLHWYQQKPGFSPKLLIYSTSNLASGVPARFSGSGSGTSYSLTISSVEAEDAATYYCQQYSGYPLTFGAGTKLELK

SEQ ID NO: 66 - protein, 108 aa, Artificial Sequence
  Humanized light chain variable region
DIQLTQSPSSMSASVGDRITITCRASSSISSNYLHWYQQKPGKSPKLLIYSTSNLASGVPSRFSGSGSGTDYTLTISSVQPEDFATYYCQQYSGYPLTFGQGTKLELK

SEQ ID NO: 67 - protein, 108 aa, Artificial Sequence
  Humanized light chain variable region
DIQLTQSPSSLSASVGDRITITCRASSSISSNYLHWYQQKPGKAPKLLIYSTSNLASGVPSRFSGSGSGTDFTLTISSVQPEDFATYYCQQYSGYPLTFGQGTKLELK

SEQ ID NO: 68 - protein, 108 aa, Artificial Sequence
  Humanized light chain variable region
DIQLTQSPSSLSASVGDRVTITCRASSSISSNYLHWYQQKPGKAPKLLIYSTSNLASGVPSRFSGSGSGTDFTLTISSLQPEDFATYYCQQYSGYPLTFGQGTKLELK

SEQ ID NO: 69 - protein, 108 aa, Artificial Sequence
  Humanized light chain variable region
DIQMTQSPSSLSASVGDRVTITCRASSSISSNYLHWYQQKPGKAPKLLIYSTSNLQSGVPSRFSGSGSGTDFTLTISSLQPEDFATYYCQQYSGYPLTFGQGTKLELK

SEQ ID NO: 70 - protein, 107 aa, Mus musculus
  Humanized light chain variable region
DIVMTQSQKFMSTSVGDRVSVTCKASQNVGTNVAWYQQKPGQSPKALIYSASYRYSGVPDRFTGSGSGTDFTLTISNVQSEDLAEYFCQQYNSYPYTFGGGTKLEIK

SEQ ID NO: 71 - protein, 106 aa, Mus musculus
  Humanized light chain variable region
DIELTQSPAIMSASPGEKVTMTCSASSSISYMHWYQQKPGTSPKRWIYDTSKLASGVPARFSGSGSGTSYSLTISRVEAEDAATYYCQQWSSNPLTFGSGTKLEIK

SEQ ID NO: 72 - protein, 106 aa, Mus musculus
  Humanized light chain variable region
DIVLTQSPAIMSASPGEKVTMTCSASSSVSYMHWYQQKSGTSPKRWIYDTSKLASGVPARFSGSGSGTSYSLTISSMEAEDAATYYCQQWSSNPLTFGAGTKLELK

SEQ ID NO: 73 - protein, 108 aa, Mus musculus
  Humanized light chain variable region
DIQMIQSPASLSASVGETVTITCRASENIYSYLAWYQQKQGKSPQLLVYNAKTLAEGVPSRFSGSGSGTQFSLKINSLQPEDFGSYYCQHHYGTPPYTFGGGTKLEIK

SEQ ID NO: 74 - protein, 107 aa, Mus musculus; identical to SEQ ID NO: 70

SEQ ID NO: 75 - protein, 107 aa, Mus musculus
DIVMTQSQKFMSTSVGDRVSVTCKASQNVGTAVAWYQQKPGQSPKLLIYSASNRYTGVPDRFTGSGSGTDFTLTISNMQSEDLADYFCQQYSSYPFTFGSGTKLEIK

SEQ ID NO: 76 - protein, 109 aa, Artificial Sequence
  Human light chain variable region
EIVLTQSPATLSLSPGERATLSCRASQSVSTYLAWYQQKPGQAPRLLIYDASNRATGIPARFSGSGSGTDFTLTISSLEPEDYAVYYCQQRSNWPPLFTFGPGTKVDIK

SEQ ID NO: 77 - protein, 109 aa, Artificial Sequence
  Human light chain variable region
EIVLTQSPATLSLSPGERATLSCRASQSVSSYLAWYQQKPGQAPRLLIYDASNRATGIPARFSGSGSGTDFTLTISSLEPEDFAVYYCQQRSNWPPSLTFGGGTKVEIK

SEQ ID NO: 78 - protein, 109 aa, Artificial Sequence
  Human light chain variable region
EIVLTQSPATLSLSPGERATLSCRASQSVSSYLAWYQQKPGQAPRLLIYDASNRATGIPARFSGSGSGTDFTLTISSLEPEDFAVYYCQQRSNWPPMYTFGQGTKLEIK

SEQ ID NO: 79 - protein, 119 aa, Mus musculus
EVQLVESGGDLVQPGGSLKLSCAASGFTFSSYGMSWVRQTPDKRLELVATINSNGGTTYYPDSVKGRFTISRDNAKHTLYLQMSSLKSEDTAMYYCTRNEEFRRGLAYWGQGTLVTVSA

SEQ ID NO: 80 - protein, 119 aa, Artificial Sequence
  Humanized heavy chain variable region
EVQLVESGGGLVQPGGSLRLSCAASGFTFSSYGMSWVRQAPGKGLELVATINSNGGTTYYPDSVKGRFTISRDNAKHTLYLQMSSLRAEDTAVYYCTRNEEFRRGLAYWGQGTLVTVSS

SEQ ID NO: 81 - protein, 119 aa, Artificial Sequence
  Humanized heavy chain variable region
EVQLVESGGGLVQPGGSLRLSCAASGFTFSSYGMSWVRQAPGKGLELVATINSNGGTTYYADSVKGRFTISRDNAKNTLYLQMSSLRAEDTAVYYCTRNEEFRRGLAYWGQGTLVTVSS

SEQ ID NO: 82 - protein, 119 aa, Artificial Sequence
  Humanized heavy chain variable region
EVQLVESGGGLVQPGGSLRLSCAASGFTFSSYGMSWVRQAPGKGLELVAAINSNGGSTYYADSVKGRFTISRDNAKNTLYLQMSSLRAEDTAVYYCTRNEEFRRGLAYWGQGTLVTVSS

SEQ ID NO: 83 - protein, 119 aa, Artificial Sequence
  Humanized heavy chain variable region
EVQLVESGGGLVQPGGSLRLSCAASGFTFSSYAMSWVRQAPGKGLELVAAINSNGGSTYYADSVKGRFTISRDNAKNTLYLQMSSLRAEDTAVYYCTRNEEFRRGLAYWGQGTLVTVSS

SEQ ID NO: 84 - protein, 121 aa, Mus musculus
  Humanized heavy chain variable region
QVQLQQSGPELVRPGVSVKISCKGSGYTFTDYAIHWAKQGHAKSLEWIGIINTYNGNSNYNQNFKGKATMTVDKSSSTAYMELTRLTSEDSAIYYCARNYGSSFNWYFDVWGQGTTLTVSS

SEQ ID NO: 85 - protein, 121 aa, Artificial Sequence
  Humanized heavy chain variable region
QVQLVQSGAEVKKPGASVKVSCKGSGYTFTDYAIHWARQAPGQGLEWIGIINTYNGNSNYAQKFQGRATMTVDKSTSTAYMELSRLRSEDTAVYYCARNYGSSFNWYFDVWGQGTTVTVSS

SEQ ID NO: 86 - protein, 121 aa, Artificial Sequence
  Humanized heavy chain variable region
QVQLVQSGAEVKKPGASVKVSCKGSGYTFTDYAIHWGRQAPGQGLEWIGIINTYNGNSNYAQKFQGRATMTRDTSTSTAYMELSRLRSEDTAVYYCARNYGSSFNWYFDVWGQGTTVTVSS

SEQ ID NO: 87 - protein, 121 aa, Artificial Sequence
  Humanized heavy chain variable region
QVQLVQSGAEVKKPGASVKVSCKASGYTFTDYAIHWGRQAPGQGLEWMGIINTYNGNSNYAQKFQGRVTMTRDTSTSTAYMELSRLRSEDTAVYYCARNYGSSFNWYFDVWGQGTTVTVSS

SEQ ID NO: 88 - protein, 124 aa, Mus musculus
QVQLQQSGPELVRPGVSVKISCKGSGYTFTDYAIHWVKQSHAKSLEWIGVINTYSGNTNYNQKFKGRATMTVDKSSSTAYMELARLTSEDSAIYFCARGVTYGSGYPYWYFDVWGAGTTVTVSS

SEQ ID NO: 89 - protein, 118 aa, Mus musculus
EVQLQQSGPELVKPGASVRISCKTSGYTFTDYVIHWVKQNHGGSLEWIGGINRDSGGTTYNQKFQDKVTLTVDKSSNTAYMELRSLTSEDSAVYYCTKWKFPWYFDVWGAGTTVTVSS

SEQ ID NO: 90 - protein, 118 aa, Mus musculus
EVQLQQSGPELVKPGASVRISCKTSGYTFTEYVIHWVKQNHGGSLEWIGGINRDSGGTTYNQKFQDKVTLTVDKSSNTAYMELRSLTSEDSAVYYCTKWKFPWYFDVWGAGTTVTVSS

SEQ ID NO: 91 - protein, 117 aa, Mus musculus
EVKLVESGGDLVKPGGSLKLSCAASGFTFSSYGMSWVRQTSDKRLEWVATISGGGRYTYYPDSVKGRFTISRDSSKNTLYLQMSSLKSEDTAMYYCVRHYDGYLDYWGLGTTLTVSS

SEQ ID NO: 92 - protein, 116 aa, Mus musculus
EVQLQESGPSLVKPSQTLSLTCSVTGDSITSGSWNWIRKFPGNKLEYMGYISYSGSIYYNPSLKSRISITRDTSKNQYYLQLNSVTTEDTATYYCARGNPAWFAYWGQGTLVTVSA

SEQ ID NO: 93 - protein, 120 aa, Mus musculus
QVQLQQSGPEVVRPGVSVKISCKGSGYTFTDYAMHWVKQSHAKSLEWIGIINTYNGNTNYNQKFKGKATMTVDKSSSTAYMEFARLTSEDSAIYYCARSRGPWDRYFDVWGAGTTVTVSS

SEQ ID NO: 94 - protein, 118 aa, Artificial Sequence
  Human heavy chain variable region
QVQLVQSGAEVKKPGSSVKVSCKASGGTFSSYAISWVRQAPGQGLEWMGGIIPILGIANYAQKFQGRVTITADESTSTAYMELSSLRSEDTAVYYCARGDSGYDSNYWGQGTLVTVSA

SEQ ID NO: 95 - protein, 119 aa, Artificial Sequence
  Human heavy chain variable region
QVQLVQSGAEVKKPGSSVKVSCKASGGTFSSYAISWVRQAPGQGLEWMGGIIPILGIANYAQKFQGRVTITADKSTSTAYMELSSLRAEDTAVYYCARGGSGRYLPDYWGQGTLVTVSA

SEQ ID NO: 96 - protein, 119 aa, Artificial Sequence
  Human heavy chain variable region
EVQLVQSGAEVKKPGSSVKVSCKASGGTFSSYAISWVRQAPGQGLEWMGGIIPIFGTANYAQKFQGRVTITADESTSTAYMELSSLRSEDTAVYYCARGERGSYLIDYWGQGTLVTVSA

SEQ ID NO: 97 - protein, 10 aa, Artificial Sequence
  CDR of heavy chain variable region
GFTFSSYAMS